European Patent Application EP 4 481 026 A1, published December 25, 2024. Title: DETERGENT COMPOSITIONS CONTAINING ENZYMES. Applicant: The Procter & Gamble Company. Application EP. The sequence listing filed with the application follows.

SEQUENCE LISTING (7 sequences)

SEQ ID NO: 1 - protein, 288 aa, Flavobacterium sp.
MSIQFSKILLLTVLATATISNAQDKKSKSKTAKIDWSHWTVTVPEENPDKPGKPYSLGYPEILNYAEDKIASKYMYDDPKDKSVVFYAFPSGVTTANTHYSRSELRETMETGSNKVNWTFAKGGKMRGTYAIDDISKEPDGKYSRVIIAQIHGVLTDEQRDLIGQKDNNAPPILKVYWDKGKIRVKTKVLKDLNAPYKEMLLEHAWGDDEGRNFKEKIDLNTRFTLEVKVSDGRMEVILNDTESLVYDDIHMKKWGIFENYFKAGNYFQSKTPGTFAKVKIYSLQVTH

SEQ ID NO: 2 - protein, 446 aa, Zobellia galactanivorans
MKKNVFTTLRTVVNGDIMWKLIPVFFLALCLGSCSEEPVDPEEEAVLTKLSANSTAIGISSVSASTSQSPNVASNTLDGSTSTRWSGYGDGASITYDLGSSANIDYVKIAFYKGDSRKTKYEVWVGNSTSSLTKIKSKTSSGSTSDYETIDLPNSTARYIRIVGKGYVLNSGGSTVLWNSITKFQAWGSGGSSTLPISGNSPASVLGITANTWKINSFIGSPGSSATYYDDITDASGISYNTYSDDNYFYTDGEWVYFKCYRGLGGSANSQNPRVELREMDNGNLASWTGDSGTHTMEWTVQVNQLPQDTDGDGGVLCFGQIHGPSKNSDGVEVDDVVRVQFIGEENQSSGSVKLKISGYVTEEQGGSQTFSGYSLDTTYNCKLVYSGGYVELFMNGSSVFRKKMEVDDLSENYFKVGNYLQSVKGASYTGSYGLVRIKNLSVTHN

SEQ ID NO: 3 - protein, 611 aa, Saccharophagus degradans
MTFIKIMGAGALIASASLANAATFVLEKVNTGFSVDGGNGAVEARQVYLWETNTNNVNQNWVQISHGGGYYSYKKQNTNLCLDGGSGGARLQPVTLEVCDSSNYDQHWNKVKVYTGTEIYRMEKRNAPGFSIDGNGGAAARQAIYLWNSNSNNVNQQWEFIRTDEDTGDGKLAIATAFDDGSSHSSYPASKAIDGNTAWASRWAASGSPVNLTIQLEQTSRVTEVGIAWGQGGSRAYTFEIYARPGTSGSWTKVFDDVSSGSTAGIEVFDITDIDAQQIRVKTFENTAGTTWTNITEVEIYGADGGSSSSSSSSSSTSSTSSTSSTSSSSGGFNLNPNAPPSSNFNLSQWYLSVPTDTDGSGTADSIKEGELNSGYENNSYFYTGSDGGMVFKCPISGYKTSTGTSYTRTELREMLRAGNTSIATSGVNKNNWVFGSAPSSAQAAAGGVDGNMKATLAVNYVTTTGDSSQVGRVIIGQIHAEKNEPIRLYYRKLPGNSKGGIYYAHEDADGGEVWVDMIGSRSSSASNPSDGIALNEVFSYEIDVTNNMLTVKIYRDGKSTVTSQYNMVNSGYDDSDDWMYFKAGVYNQNNTGNGSDYVQATFYSLTHTHD

SEQ ID NO: 4 - protein, 307 aa, Klebsiella pneumoniae
MLKSGVMVASLCLFSVPSRAAVPAPGDKFELSGWSLSVPVDSDNDGKADQIKEKTLAAGYRNSDFFTLSDAGGMVFKAPISGAKTSKNTTYTRSELREMLRKGDTSIATQGVSRNNWVLSSAPLSEQKKAGGVDGTLEATLSVDHVTTTGVNWQVGRVIIGQIHANNDEPIRLYYRKLPHHQKGSVYFAHEPRKGFGDEQWYEMIGTLQPSHGNQTAAPTEPEAGIALGETFSYRIDATGNKLTVTLMREGRPDVVKTVDMSKSGYSEAGQYLYFKAGVYNQNKTGKPDDYVQATFYRLKATHGAQR

SEQ ID NO: 5 - protein, 248 aa, Zobellia galactanivorans
GNSPASVLGITANTWKINSFIGSPGSSATYYDDITDASGISYNTYSDDNYFYTDGEWVYFKCYRGLGGSANSQNPRVELREMDNGNLASWTGDSGTHTMEWTVQVNQLPQDTDGDGGVLCFGQIHGPSKNSDGVEVDDVVRVQFIGEENQSSGSVKLKISGYVTEEQGGSQTFSGYSLDTTYNCKLVYSGGYVELFMNGSSVFRKKMEVDDLSENYFKVGNYLQSVKGASYTGSYGLVRIKNLSVTHN

SEQ ID NO: 6 - protein, 260 aa, Flavobacterium sp.
RNGANIDLSHWTLTTPAEDPKKPGKTFDLNYPEIFDFASNDIAKKYMYEDPKDKSIVFYAYPSGTSTANSHFSRSELRETMEIGSKNVNWTFAQGGYFKGTYAIEDVSKEADGKYSRVIIAQIHGILTDSQQALIGQKDKNAAPILKIFWDQGKIRVKTKVLKNQNASLKEMLPADAWTDDKGRDFKEKIDFNTKFTLEIKVSDGRLEVIMNGTESFVYEDINIKKWGVFENYFKAGNYFQSTNPNTFAKVKIYDLQVSH

SEQ ID NO: 7 - protein, 391 aa, Flavobacterium sp.
KLVTTKLTPASVSDNGNDGNVAANTLDGNLSTRWSSDGSTGKYITYDLGSSKSISSLKIAWHQGDQRKSYFQIRVGDSTGSLTTVYDAKTTGSSGTTTALETYTLSSPVTARYVRISCFGNSLTTWNSIAETEIYSTVDDGLPDTYPTSVIGITANTWKINSFTGTPGSSAVYYDDITTASGVSYNTYNDPNYFYTDGTWTYFKCYRGLGTSSNSSNPRVELRELNNGSSASWDGSVGTHTMTWTVKVDKLPKGENGTTGVLCFGQIHGPSTNSSGVAVDDIIRVQFDGAANQSTGTVKLKISGYITEKVLGGSKSFTGYSLGTSYTFTIKYTGGKVYLYNGSTLVFSQQMDTSTEGNYFKAGNYLQSVKNVSYDGSYGLVGISSLTVSHQ